European Patent Specification EP 3 442 326 B1, published December 11, 2024. Title: TOBACCO PLANTS EXHIBITING ALTERED PHOTOSYNTHESIS AND METHODS OF MAKING AND USING. Applicant: ALTRIA CLIENT SERVICES LLC. The sequence listing filed with the application follows.

SEQUENCE LISTING (56 sequences)

SEQ ID NO: 1 - DNA, 25 bp, Artificial Sequence
  source: /note="Description of Artificial Sequence: Synthetic primer"
atggcttctctattatcttctcgtc

SEQ ID NO: 2 - DNA, 24 bp, Artificial Sequence
  source: /note="Description of Artificial Sequence: Synthetic primer"
tcatgggaagatagcattaacaaa

SEQ ID NO: 3 - DNA, 28 bp, Artificial Sequence
  source: /note="Description of Artificial Sequence: Synthetic primer"
atggcttctctattatcttctcgtctcc

SEQ ID NO: 4 - DNA, 25 bp, Artificial Sequence
  source: /note="Description of Artificial Sequence: Synthetic primer"
ttaaatagaatctgccacataaatg

SEQ ID NO: 5 - DNA, 26 bp, Artificial Sequence
  source: /note="Description of Artificial Sequence: Synthetic primer"
atggatgctctcttcgtcaattcctc

SEQ ID NO: 6 - DNA, 23 bp, Artificial Sequence
  source: /note="Description of Artificial Sequence: Synthetic primer"
gcccttgttcaacttactacatt

SEQ ID NO: 7 - DNA, 25 bp, Artificial Sequence
  source: /note="Description of Artificial Sequence: Synthetic primer"
atggatgctctgttcgtcaattcct

SEQ ID NO: 8 - DNA, 25 bp, Artificial Sequence
  source: /note="Description of Artificial Sequence: Synthetic primer"
tcaacttactacattctgttgaccc

SEQ ID NO: 9 - DNA, 27 bp, Artificial Sequence
  source: /note="Description of Artificial Sequence: Synthetic primer"
atggaagccactgcttctttctcctca

SEQ ID NO: 10 - DNA, 26 bp, Artificial Sequence
  source: /note="Description of Artificial Sequence: Synthetic primer"
ttagttcttggccccaaaaccacgag

SEQ ID NO: 11 - DNA, 1116 bp, Nicotiana tabacum
atggcttctctattatcttctcgtctcccacgtcatctttcctctaataaaccggtactcccaccatcaagctccggttcaaatctccttcacaacttcacatataaaacccggttcgatcaatcccggttcaaatgctcagctggtggaacggggttcttcacgaagttgggtcgtttgctgaaagagaaagcaaagagcgacgtggagaaactgttctcaggattctcaaaaactcgagacaatttagcagttatagatgaactcctcctttactggaacctttctgacactgaccgtgttcttgatgaacttgaagaggttctgttggtgtctgattttggcccgaagattaccataaagattgtggagagcttgcgggaggatatatatggggggaaaatcaaatcaggaagtgagattaaaagtgctcttaagaagagtatcttggatctattgactagcaaggcacctaaaacagagctccgtctgggcttcaggaaaccatctgtgatcatgattgtgggcgtcaacggaggtgggaagacaacatctcttggaaagctggcaaatagattgaagaaagaaggggctaagatactattagcagctggtgatacatttagagcagctgctagtgatcagttagaaatttgggctgaaaggactggttgtgagatcgttgttgctgaaaaagagaaagctaaggcatcatcagttctttcgcaggctgttaaaagaggaaaggaagagggtttcgatattgttttatgcgacacatctggccgtctgcacacctactatagcttgatggaggaattggtggcatgcaaaaaagttgtcagtaaaattgttactggtgcacctaatgaaatcttgcttgtactggatggaactactggtttaaatatgcttccacaagcaagagagtttaacgatgttgttggagtcactggcttaatattgactaaacttgatggttctgctcgaggtggctgtgtggttagtgtggttgatgaacttggcattcctgtaaagtttgtaggtgttggggaaggtgtagatgacctccaaccgttcaatgctgaggaatttgttaatgctatcttcccatga

SEQ ID NO: 12 - protein, 371 aa, Nicotiana tabacum
MASLLSSRLPRHLSSNKPVLPPSSSGSNLLHNFTYKTRFDQSRFKCSAGGTGFFTKLGRLLKEKAKSDVEKLFSGFSKTRDNLAVIDELLLYWNLSDTDRVLDELEEVLLVSDFGPKITIKIVESLREDIYGGKIKSGSEIKSALKKSILDLLTSKAPKTELRLGFRKPSVIMIVGVNGGGKTTSLGKLANRLKKEGAKILLAAGDTFRAAASDQLEIWAERTGCEIVVAEKEKAKASSVLSQAVKRGKEEGFDIVLCDTSGRLHTYYSLMEELVACKKVVSKIVTGAPNEILLVLDGTTGLNMLPQAREFNDVVGVTGLILTKLDGSARGGCVVSVVDELGIPVKFVGVGEGVDDLQPFNAEEFVNAIFP

SEQ ID NO: 13 - DNA, 966 bp, Nicotiana tabacum
atggcttctctattatcttctcgtctcccacatcatctttcctctaataaaccggtactcccaccatcaagctccggttcaaatctccttcacaacttcacatataaaacccggttcgatcaatcccggttcaaatgctcagctggtggaacggggttcttcacgaagttgggtcgtttgctgaaagagaaagcaaagagcgacgtggagaaactgttctcaggattctcaaaaactcgagacaatttagcagttatagatgaactcctcctttactggaacctttctgacactgaccgtgttcttgatgaacttgaagaggttctgttggtgtctgattttggcccgaagattaccataaagattgtggagagcttgcgggaggatatatatggggggaaaatcaaatcaggaagtgagattaaaagtgctcttaagaagagtatcttggatctattgactagcaaggcacctaaaacagagctccgtctgggcttcaggaaaccatctgtgatcatgattgtgggcgtcaacggaggtgggaagacaacatctcttggaaagctggcaaatagattgaagaaagaaggggctaagatactattagcagctggtgatacatttagagcagctgctagtgatcagttagaaatttgggctgaaaggactggttgtgagatcgttgttgctgaaaaagagaaagctaaggcatcatcagttctttcgcaggctgttaaaagaggaaaggaagagggtttcgatattgttttatgcgacacatctggccgtctgcacacctactatagcttgatggaggaattggtggcatgcaaaaaagttgtcagtaaaattgttactggtgcacctaataggagcagtatacaacaggaactaagattagcagcttgctactactctgaaaattcaacattcacaaataacatttatgtggcagattctatttaa

SEQ ID NO: 14 - protein, 320 aa, Nicotiana tabacum
MASLLSSRLPHHLSSNKPVLPPSSSGSNLLHNFTYKTRFDQSRFKCSAGGTGFFTKLGRLLKEKAKSDVEKLFSGFSKTRDNLAVIDELLLYWNLSDTDRVLDELEEVLLVSDFGPKITIKIVESLREDIYGGKIKSGSEIKSALKKSILDLLTSKAPKTELRLGFRKPSVIMIVGVNGGGKTTSLGKLANRLKKEGAKILLAAGDTFRAAASDQLEIWAERTGCEIVVAEKEKAKASSVLSQAVKRGKEEGFDIVLCDTSGRLHTYYSLMEELVACKKVVSKIVTGAPNRSSIQQELRLAACYYSENSTFTNNIYVADS

SEQ ID NO: 15 - DNA, 1121 bp, Nicotiana tabacum
atggatgctctcttcgtcaattcctctctctcccgcctcaaactcaaattctcccctcaattccctcccaccttctctcatcaaccttttatctgtctaaagaaactcggcaataagaacaatttatcagtatttgctacgcttcagaaccagcagcaacaagcagtcgaagcagcagaagacgaagaaccggtactgtttgaagattacgatgaggatgaaacgtacggagaagttaacaaaattatcggcagtcgagcaattgaacgtgggaaaggaatggagtacttgatagagtggaaagacgaacatgccccaacgtgggtcccctctgattacattgctaaagatgttgtggccgagtacgaaactccttggtggaatgcggctaaaaaggccgacgaatccgctcttagggaactcctagaaactgacgacgacagagatgtggacgcagtagatgaggatggacgtacggctttgctctttgtctcgggtctggggtccgagccgtgtgtcaagctgctagctgaagccggcgctgacgtggactatcgcgataggaatggcggcttgactgctctgcatatggcagccggctatgttaagccgggtgtcgccaagctgttaattgacctcggggcagaccccgaggtcgaggattatagaggacaaacgcctctgagcttggcgaggatgattttgaatcaaacgcctaaaggaaatccaatgcaattcgcgaggagattggggttagagaatgtggttaggattttggaggatgcgattttcgagtatgcaacagtggaggaaatattggagaagagagggaaaggcgaaaatgtggagtatttagtgaagtggaaggatggggaggataacgagtgggtcaaagcatggctgatatctgaagatttggtgagggattttgaggctggtttggaatatgcagtagcagattgtattcttgagaagagagaaggtgaggatgggaagggagaatacttggttaaatggactgatattgaggaagctacgtgggaacccgaagaaaatgttgacccccttcttatagaagattttgaaaagagtcaacagaatgtagtaagttgaacaagggc

SEQ ID NO: 16 - protein, 370 aa, Nicotiana tabacum
MDALFVNSSLSRLKLKFSPQFPPTFSHQPFICLKKLGNKNNLSVFATLQNQQQQAVEAAEDEEPVLFEDYDEDETYGEVNKIIGSRAIERGKGMEYLIEWKDEHAPTWVPSDYIAKDVVAEYETPWWNAAKKADESALRELLETDDDRDVDAVDEDGRTALLFVSGLGSEPCVKLLAEAGADVDYRDRNGGLTALHMAAGYVKPGVAKLLIDLGADPEVEDYRGQTPLSLARMILNQTPKGNPMQFARRLGLENVVRILEDAIFEYATVEEILEKRGKGENVEYLVKWKDGEDNEWVKAWLISEDLVRDFEAGLEYAVADCILEKREGEDGKGEYLVKWTDIEEATWEPEENVDPLLIEDFEKSQQNVVS

SEQ ID NO: 17 - DNA, 1113 bp, Nicotiana tabacum
atggatgctctgttcgtcaattcctctctctcccgcctcaaactcaaattctcccctcaattccctcccaccttctctcatcaaccttttatccgtctaaagaaactcggcaacaagaacaatttctcagtatttgctacgcttcagaaccagcagcaacaagcagtcgcagctgctgaagaggaagaaccggtactgtttgaagattacgatgaggatgaaacgtacggagaagttaacaaaatcatcggaagtagagcaattgaaggtgggaaaggaatggagtacttgatagagtggaaagacgaacatgccccaacatgggtcccctctgattacattgctaaagatgttgtggccgagtacgaaactccttggtggaatgccgctaaaaaggccgacgaatccgctcttaagaaatttctagaagctgacgacgacagagatgtggacgcagttgatgaggatggacgtacggctttgctctttgtctcgggtctggggtccgagccgtgtgtcaagctgctagctgaagctggcgctgacgtggactatcgcgataggaatggcggcttgacggctctgcacatggcagccggctatgttaagccgggtgtcgccaagctgttaattgacctcggggcagaccctgaggtcgaggattatagaggacaaacgcctctgagcttggcgaggatgattttgaatcaaacgcctaaaggaaacccaatgcaatttgctaggagattgggactagagaatgtggttaggatattggaggatgcgattttcgaatatgcaacagtggaggagatattggagaagagagggaaaggtgaaaatgtggagtatttagtcaagtggaaggatggggaggataatgaatgggtgaaagcatggctgataagtgaggatttggtgagagattttgaggctggtttggaatatgcagtggcagagtgtattcttgagaagagagaaggtgaggatgggaagggagaatatttggttaaatggactgatattgaggaagctacctgggaaccggaagaaaatgttgacccccttctaatagaagattttgaaaagggtcaacagaatgtagtaagttga

SEQ ID NO: 18 - protein, 370 aa, Nicotiana tabacum
MDALFVNSSLSRLKLKFSPQFPPTFSHQPFIRLKKLGNKNNFSVFATLQNQQQQAVAAAEEEEPVLFEDYDEDETYGEVNKIIGSRAIEGGKGMEYLIEWKDEHAPTWVPSDYIAKDVVAEYETPWWNAAKKADESALKKFLEADDDRDVDAVDEDGRTALLFVSGLGSEPCVKLLAEAGADVDYRDRNGGLTALHMAAGYVKPGVAKLLIDLGADPEVEDYRGQTPLSLARMILNQTPKGNPMQFARRLGLENVVRILEDAIFEYATVEEILEKRGKGENVEYLVKWKDGEDNEWVKAWLISEDLVRDFEAGLEYAVAECILEKREGEDGKGEYLVKWTDIEEATWEPEENVDPLLIEDFEKGQQNVVS

SEQ ID NO: 19 - DNA, 1692 bp, Nicotiana tabacum
atggaagccactgcttctttctcctcaactatgtcttcccaccatttctttccactttccaaagccaccctctcaacttctaaacttccattttctgggactggttcaactcattctctttcattttcttcaagaaactcattcactagggatacatggagggtgatcaattcaaggaatgtggttatttcaagaagagaaatgcgtggagttattagagctgagatgtttggacagctcactagtggacttgaatcagcttggaataagctcaaaggagaagaggttttgaccaaggaaaacattgtggaacctatgagagacatcaggagggctcttttggaagctgatgttagtctccctgttgtcagaaggtttgttcagtctgttagtgacgaagccgtggggactggcttgattcgaggagtaagaccagatcagcaactagttaaaattgtacgagacgagcttgtgaaactgatgggtggagaggtctctgaactggtatttgctaaatctggacccaccataatactattggccggtctacaaggtgttggaaagacaactgttagcgcaaagttagctttatatctaaagaagcagggtaagagttgcatgctgattgctggagacgtgtatagacctgctgctattgaccaacttgttattttgggtgaacaggttgatgtgcctgtttatgcagcaggaacagacgtaaaacctgcagaaatagcccgtcaaggattagaagaggccaaaagaaagaatgtagatgtagtcataatggatacagctggacgacttcagatagataaagctatgatggatgaattaaaagaggtgaaacgggtactgaaccccacagaggttttgcttgttgtggatgcaatgactggccaagaagctgcagctttggtcacaacattcaatctcgaaattggaattactggtgccattatgacaaagctagatggggattctaggggtggagcagctttaagtgtcaaggaggtatcaggaaagccaattaagctcgtaggaagaggtgaacgtatggaggaccttgaacctttctatcctgaccgcatggctggacgtattttagggatgggagatgttctgtcgtttgttgaaaaagcccaagaagttatgaaacaagaagatgcagaagatttgcagaagaagatcatgagtgcaaaatttgatttcaatgacttcctgaagcaaactcgtgcagttgctcaaatgggtaccatgtcccgcgttctcggaatgattcctggcatgggaaaggttactcctgcacaaattcgagaggcagagaagagcttaataataatggagtcaatgatagaagtcatgacaccagaggagaaggagaaaccagaactgttagcagaatctcctagtagaaggaaacgtattgctcaagagtccgggaaaactgagcagcaggtgagtcaacttgttgctcaactttttcaaatgcgtgtacgtatgaagaatttgatgggtgttatgcaaggtggttccatacctgcactgagtaatcttgaggaggcacttaaaactgaacagaaggctcctcctggtactgcaaggaggaagcgaaggtcagaatcaagaaagcaatttgcagactcgggatcaactagacctggccctcgtggttttggggccaagaactaa

SEQ ID NO: 20 - protein, 563 aa, Nicotiana tabacum
MEATASFSSTMSSHHFFPLSKATLSTSKLPFSGTGSTHSLSFSSRNSFTRDTWRVINSRNVVISRREMRGVIRAEMFGQLTSGLESAWNKLKGEEVLTKENIVEPMRDIRRALLEADVSLPVVRRFVQSVSDEAVGTGLIRGVRPDQQLVKIVRDELVKLMGGEVSELVFAKSGPTIILLAGLQGVGKTTVSAKLALYLKKQGKSCMLIAGDVYRPAAIDQLVILGEQVDVPVYAAGTDVKPAEIARQGLEEAKRKNVDVVIMDTAGRLQIDKAMMDELKEVKRVLNPTEVLLVVDAMTGQEAAALVTTFNLEIGITGAIMTKLDGDSRGGAALSVKEVSGKPIKLVGRGERMEDLEPFYPDRMAGRILGMGDVLSFVEKAQEVMKQEDAEDLQKKIMSAKFDFNDFLKQTRAVAQMGTMSRVLGMIPGMGKVTPAQIREAEKSLIIMESMIEVMTPEEKEKPELLAESPSRRKRIAQESGKTEQQVSQLVAQLFQMRVRMKNLMGVMQGGSIPALSNLEEALKTEQKAPPGTARRKRRSESRKQFADSGSTRPGPRGFGAKN

SEQ ID NO: 21 - DNA, 1605 bp, Nicotiana tabacum
atgtccgccattgctacttctgctgctctctcttttcctttctctttctgccgttctaccaagacttttgctacaagaaagtgtttcaaagggggatttggagtgtttgcagtgtatgaggaggcaggtgagttaacaaacaagaaaagctcctggttgacactctttgatgtggaagatccaaggtcaaaatttcctcagtctaaaggcaagttcctggatgcaaatcaagctttagaagttgctagatttgatatacaatattgtgattggcgagctcggcaagatgtattaaccataatgctcctgcacgaaaaggttgtggaagtattgaatcctctggcacgtgagtacaaatctattggaaccatgaagaaggaactagcagagttacaaggagcactttctcaggctcataaagaggtacatatatctgaggtgcgggtttctgctgctttagataagctagctcacatggaagcattggttaatgataggctgcttccggagaggagtgcagaagaatcagattgcccgtcttcctccaccggtacgtctacagtatctagagatactgttaaaggcaagcagcctaggagaaccctcaatgtgtcaggtccggtccaagattacagctctcatttgaagaacttttggtatcctgtcgctttttctgctgatgttaaggaagacacaatgacaccaattgattgctttgaggaaccatgggtgatttttcgtgggaaagatggaaaacctggatgtgtccggaacacatgtgcacatagagcctgcccccttcatttgggttcagttaatgagggtcgcatccaatgtccttatcatgggtgggaatattcaacagacggaaaatgtgagaaaatgccatcaactaaatttctgaatgtcaagatcaaagctctgccatgctttgagcaagagggaatgatatggatttggcctggaaatgatcctcctgcagctactcttccttctttactgccaccttctggatttcaaatccatgcagagattgttattgaacttccagtggaacatgggctacttttggacaatctgttggatcttgcacatgctcctttcacccatacgtctacatttgctaaaggatggactgtcccaagctttgtaaaatttttgactcctgcatctggtcttcaaggatattgggatccctatccaatagatatggaatttcgaccaccttgtatagttctatcaaccattggaatctcaaagccaggcaagttggaagggcagagtaccaaagagtgctctacacacctacaccaacttcatgtatgtttacctgcatctaaacagaagacaaggttgttatataggatgtcactggattttgctcccgtgctaaaacacatccctttcatgcaatacgtgtggaggcattttgctgaacaggttttaaacgaagacctacggcttgtgattggtcagcaagagcggatgctcaatggtgctaacatttggaacctgcctgtgtcatacgataagctaggagtgaggtataggatatggagagatgctgtagagagtggagcaaagcaattgccattcagcaaatga

SEQ ID NO: 22 - protein, 534 aa, Nicotiana tabacum
MSAIATSAALSFPFSFCRSTKTFATRKCFKGGFGVFAVYEEAGELTNKKSSWLTLFDVEDPRSKFPQSKGKFLDANQALEVARFDIQYCDWRARQDVLTIMLLHEKVVEVLNPLAREYKSIGTMKKELAELQGALSQAHKEVHISEVRVSAALDKLAHMEALVNDRLLPERSAEESDCPSSSTGTSTVSRDTVKGKQPRRTLNVSGPVQDYSSHLKNFWYPVAFSADVKEDTMTPIDCFEEPWVIFRGKDGKPGCVRNTCAHRACPLHLGSVNEGRIQCPYHGWEYSTDGKCEKMPSTKFLNVKIKALPCFEQEGMIWIWPGNDPPAATLPSLLPPSGFQIHAEIVIELPVEHGLLLDNLLDLAHAPFTHTSTFAKGWTVPSFVKFLTPASGLQGYWDPYPIDMEFRPPCIVLSTIGISKPGKLEGQSTKECSTHLHQLHVCLPASKQKTRLLYRMSLDFAPVLKHIPFMQYVWRHFAEQVLNEDLRLVIGQQERMLNGANIWNLPVSYDKLGVRYRIWRDAVESGAKQLPFSK

SEQ ID NO: 23 - DNA, 1605 bp, Nicotiana tabacum
atgtccgccattgctacttctgctgctctctcttttcctttctctttttgccgttctaccaagacttttactacaagaaagtgtttcaaagggggatttggagtgtttgcagtgtatgaggaggcaggtgagttaacaaacaagaaaagctcctggttgacactctttgatgtggaagatccaaggtcaaaatttcctcagtctaaaggcaagttcctggatgcaaatcaagctttagaagttgctagatttgatatgcaatattgtgattggcgagctcggcaagacgtacttacaataatgctcctgcatgaaaaggttgtggaagtattgaatcctctagctcgtgaatataaatctattggaaccatgaagaaggaactcgcggagttacaagaagaactgtctcgggctcacaaagaggtacatatatctgaggtgcgggtttctgctgctttagataagctagctcacatggaagcattggttaatgataggctgcttccggagaggagtacagaagaatcagattccccatcttcctccaccggtacgtctacagtatctagagataatgctaaaagcaagcagcctaggagaaccctcaatgtgtcaggtcccgtccaagattacagctcctatttgaagaacttttggtatcctgtggctttttctgctgatgttaaggaagataccatgacaccaattgattgctttgaggaaccgtgggtgatttttcgtgggaaagatggaaaacctggatgtgtccagaacacatgtgcacatagagcttgcccccttcatttgggttcagtgaatgagggtcgcatacaatgtccttatcacgggtgggaatattcaacagacggaaaatgtgagaaaatgccatcaacaaaatttctgaatgtcaagatcaaagctctgccatgctttgagcaagagggaatgatatggatttggcctggaaacgatcctcctgcagctactcttccttctttgctaccaccttctggatttcaaatccatgcagagattgtcatggaacttccggtggaacatgggctacttttggacaatctgttggatcttgcacatgctcctttcactcatacgtctacatttgctaaaggatggactgtcccaagctttgtaaaatttttgactcctgcgtctggtctgcaaggatattgggatccatatccaatagatatggaatttcgaccgccttgtatggttctgtcaaccattggaatctcaaagccgggcaaattggaagggcagagtatcaaagagtgctctacacaccttcaccaacttcatgtatgtttacctgcatctaaacagaagacaaggttgttatataggatgtcactggattttgctcctgttctaaaacacatccctttcatgcaatacgtgtggaggcattttgctgaacaggttttaaatgaagacctacggcttgtgattggtcagcaagaacggatgctcaatggtgctaacatttggaacctgcctgtgtcatacgataagctaggagtgaggtatagaatatggagagacgctgtagagagtggagcaaagcagttgccgttcagcaaatga

SEQ ID NO: 24 - protein, 534 aa, Nicotiana tabacum
MSAIATSAALSFPFSFCRSTKTFTTRKCFKGGFGVFAVYEEAGELTNKKSSWLTLFDVEDPRSKFPQSKGKFLDANQALEVARFDMQYCDWRARQDVLTIMLLHEKVVEVLNPLAREYKSIGTMKKELAELQEELSRAHKEVHISEVRVSAALDKLAHMEALVNDRLLPERSTEESDSPSSSTGTSTVSRDNAKSKQPRRTLNVSGPVQDYSSYLKNFWYPVAFSADVKEDTMTPIDCFEEPWVIFRGKDGKPGCVQNTCAHRACPLHLGSVNEGRIQCPYHGWEYSTDGKCEKMPSTKFLNVKIKALPCFEQEGMIWIWPGNDPPAATLPSLLPPSGFQIHAEIVMELPVEHGLLLDNLLDLAHAPFTHTSTFAKGWTVPSFVKFLTPASGLQGYWDPYPIDMEFRPPCMVLSTIGISKPGKLEGQSIKECSTHLHQLHVCLPASKQKTRLLYRMSLDFAPVLKHIPFMQYVWRHFAEQVLNEDLRLVIGQQERMLNGANIWNLPVSYDKLGVRYRIWRDAVESGAKQLPFSK

SEQ ID NO: 25 - DNA, 1596 bp, Nicotiana tabacum
atgacagccattactactgctctttcttttcctttctctttgtgccgctctactaagtcttatactagaaagtatgtcaaagggagctttggagtgtttgcagtatatggggaggagggtgggatgccagataagaaaagttcctggttgacactctttaatgtggaagatccaaggtctaaagttccacaaattaaaggcaaattcttggatgcaaatcaagctttggaagttgctagatatgatctacaatactgtgattggcgagctcggcaagatgtacttacaatcatgctgctgcatgaaaaggttgtggaagtgttgaaccctctagcacgtgaatacaaatctattggaaccatgaaaaaggaacttgcagagttgcaaggagagctttctcaggcccacaaccaggtacatatatctgaggcccgggtttctgctgctttggataagctagcttacatggaagagttggttaatgataggcttctgcaagagagaagcacggcagaatcagattgctcgtcctcctctgccagtacgtcaacagcattattggatactgttaaaagcaagcaaccccgaagaaccctgagtgtgtcaggtcctgtccaagattacagttcccgtttgaagaacttttggtaccctgttgctttctccgcagatcttaaggatgacaccatgttaccgattgattgctttgagcaaccatgggtgatctttcgcgggaatgatggaaaacctggatgtgtacagaatacgtgtgcacatagagcctgcccccttgatcttggctcagtgaaagagggacgcattcagtgcccttatcacggatgggaatactcaactgatgggaagtgtgagaaaatgccatcaacacgattactgaatgtaaagatcaaagcactgccctgctttgagcaagagggaatgatatggatttggccaggaaatgatccccctgcagctacccttccttctttactaccgccttctggatttcaaatccatgcggagatagtcatggaacttccagtggaacatgggctattattagacaatttattggatcttgcacatgctcctttcacccatacatcaacctttgctaaaggatggagtgtcccaagattggtgaagtttttgactcctgcttctggtctgcaaggatattgggatccttatccaatagatatggaatttagaccaccttgtatggttttatcaaccattggaatctcaaagccaggcaaattggaggggcagagtaccaagcagtgttgtacacaccttcatcaacttcatgtttgcttacctgcatcacgacacaagacacggttattatataggatgtcactggattttgctcccctgctgaaacacatccctttcatgcaatatgtttggagacattttgccgaacaggttttaaatgaagacctacggcttgtgttgggccagcaggatcgcatgctcaatggcgccaatatttggaacttgccagtgtcttacgataagctaggtgtgaggtatagaatatggagagatgctgtagatagtggagcaaagcatctaccattcagcaaataa

SEQ ID NO: 26 - protein, 531 aa, Nicotiana tabacum
MTAITTALSFPFSLCRSTKSYTRKYVKGSFGVFAVYGEEGGMPDKKSSWLTLFNVEDPRSKVPQIKGKFLDANQALEVARYDLQYCDWRARQDVLTIMLLHEKVVEVLNPLAREYKSIGTMKKELAELQGELSQAHNQVHISEARVSAALDKLAYMEELVNDRLLQERSTAESDCSSSSASTSTALLDTVKSKQPRRTLSVSGPVQDYSSRLKNFWYPVAFSADLKDDTMLPIDCFEQPWVIFRGNDGKPGCVQNTCAHRACPLDLGSVKEGRIQCPYHGWEYSTDGKCEKMPSTRLLNVKIKALPCFEQEGMIWIWPGNDPPAATLPSLLPPSGFQIHAEIVMELPVEHGLLLDNLLDLAHAPFTHTSTFAKGWSVPRLVKFLTPASGLQGYWDPYPIDMEFRPPCMVLSTIGISKPGKLEGQSTKQCCTHLHQLHVCLPASRHKTRLLYRMSLDFAPLLKHIPFMQYVWRHFAEQVLNEDLRLVLGQQDRMLNGANIWNLPVSYDKLGVRYRIWRDAVDSGAKHLPFSK

SEQ ID NO: 27 - DNA, 723 bp, Artificial Sequence
  source: /note="Description of Artificial Sequence: Synthetic polynucleotide"
ggatccatggcttctctattatcttctcgtctcccacgtcatctttcctctaataaaccggtactcccaccatcaagctccggttcaaatctccttcacaacttcacatataaaacccggttcgatcaatcccggttcaaatgctcagctggtggaacggggttcttcacgaagttgggtcgtttgctgaaagagaaagcaaagagcgacgtggagaaactgttctcaggattctcaaaaactcgagacaatttagcagttatagatgaactcctcctttactggtaataagatcttcaacacctacaccatttttttaatcactactacccattgcattgaacaaacttccaagttcttcttagcttcagattaagaaagtaccctttcttggctttgttgatgtggtaccattgtccattgtcttgtgtgtttccaccagtaaaggaggagttcatctataactgctaaattgtctcgagtttttgagaatcctgagaacagtttctccacgtcgctctttgctttctctttcagcaaacgacccaacttcgtgaagaaccccgttccaccagctgagcatttgaaccgggattgatcgaaccgggttttatatgtgaagttgtgaaggagatttgaaccggagcttgatggtgggagtaccggtttattagaggaaagatgacgtgggagacgagaagataatagagaagccattctaga

SEQ ID NO: 28 - DNA, 765 bp, Artificial Sequence
  source: /note="Description of Artificial Sequence: Synthetic polynucleotide"
ggatccgggaaaggaatggagtacttgatagagtggaaagacgaacatgccccaacgtgggtcccctctgattacattgctaaagatgttgtggccgagtacgaaactccttggtggaatgcggctaaaaaggccgacgaatccgctcttagggaactcctagaaactgacgacgacagagatgtggacgcagtagatgaggatggacgtacggctttgctctttgtctcgggtctggggtccgagccgtgtgtcaagctgctagctgaagccggcgctgacgtggactatcgcgataggaatggctaataagatcttcaacacctacaccatttttttaatcactactacccattgcattgaacaaacttccaagttcttcttagcttcagattaagaaagtaccctttcttggctttgttgatgtggtaccattgtccattgtcttgtgtgtttccagccattcctatcgcgatagtccacgtcagcgccggcttcagctagcagcttgacacacggctcggaccccagacccgagacaaagagcaaagccgtacgtccatcctcatctactgcgtccacatctctgtcgtcgtcagtttctaggagttccctaagagcggattcgtcggcctttttagccgcattccaccaaggagtttcgtactcggccacaacatctttagcaatgtaatcagaggggacccacgttggggcatgttcgtctttccactctatcaagtactccattcctttccctctaga

SEQ ID NO: 29 - DNA, 747 bp, Artificial Sequence
  source: /note="Description of Artificial Sequence: Synthetic polynucleotide"
ggatccatggaagccactgcttctttctcctcaactatgtcttcccaccatttctttccactttccaaagccaccctctcaacttctaaacttccattttctgggactggttcaactcattctctttcattttcttcaagaaactcattcactagggatacatggagggtgatcaattcaaggaatgtggttatttcaagaagagaaatgcgtggagttattagagctgagatgtttggacagctcactagtggacttgaatcagcttggaataagctcaaaggagaagaggttttgtaataagatcttcaacacctacaccatttttttaatcactactacccattgcattgaacaaacttccaagttcttcttagcttcagattaagaaagtaccctttcttggctttgttgatgtggtaccattgtccattgtcttgtgtgtttccacaaaacctcttctcctttgagcttattccaagctgattcaagtccactagtgagctgtccaaacatctcagctctaataactccacgcatttctcttcttgaaataaccacattccttgaattgatcaccctccatgtatccctagtgaatgagtttcttgaagaaaatgaaagagaatgagttgaaccagtcccagaaaatggaagtttagaagttgagagggtggctttggaaagtggaaagaaatggtgggaagacatagttgaggagaaagaagcagtggcttccattctaga

SEQ ID NO: 30 - DNA, 987 bp, Artificial Sequence
  source: /note="Description of Artificial Sequence: Synthetic polynucleotide"
ggatccgaggcaggtgagttaacaaacaagaaaagctcctggttgacactctttgatgtggaagatccaaggtcaaaatttcctcagtctaaaggcaagttcctggatgcaaatcaagctttagaagttgctagatttgatatacaatattgtgattggcgagctcggcaagatgtattaaccataatgctcctgcacgaaaaggttgtggaagtattgaatcctctggcacgtgagtacaaatctattggaaccatgaaaaaggaacttgcagagttgcaaggagagctttctcaggcccacaaccaggtacatatatctgaggcccgggtttctgctgctttggataagctagcttacatggaagagttggttaatgataggcttctgcaagagagaagcacggcagaatcagattaataagatcttcaacacctacaccatttttttaatcactactacccattgcattgaacaaacttccaagttcttcttagcttcagattaagaaagtaccctttcttggctttgttgatgtggtaccattgtccattgtcttgtgtgtttccaatctgattctgccgtgcttctctcttgcagaagcctatcattaaccaactcttccatgtaagctagcttatccaaagcagcagaaacccgggcctcagatatatgtacctggttgtgggcctgagaaagctctccttgcaactctgcaagttcctttttcatggttccaatagatttgtactcacgtgccagaggattcaatacttccacaaccttttcgtgcaggagcattatggttaatacatcttgccgagctcgccaatcacaatattgtatatcaaatctagcaacttctaaagcttgatttgcatccaggaacttgcctttagactgaggaaattttgaccttggatcttccacatcaaagagtgtcaaccaggagcttttcttgtttgttaactcacctgcctctctaga

SEQ ID NO: 31 - DNA, 3155 bp, Artificial Sequence
  source: /note="Description of Artificial Sequence: Synthetic polynucleotide"
  misc_feature (1)..(480): /note="pCSVMV Promoter"
  misc_feature (523)..(551): /note="Cloning region"
  misc_feature (601)..(840): /note="NOS terminator"
  misc_feature (841)..(1980): /note="ACTII Promoter"
  misc_feature (2101)..(2820): /note="NPT II Kan Resistance"
  misc_feature (2941)..(3120): /note="NOS Terminator"
aagcttccagaaggtaattatccaagatgtagcatcaagaatccaatgtttacgggaaaaactatggaagtattatgtgagctcagcaagaagcagatcaatatgcggcacatatgcaacctatgttcaaaaatgaagaatgtacagatacaagatcctatactgccagaatacgaagaagaatacgtagaaattgaaaaagaagaaccaggcgaagaaaagaatcttgaagacgtaagcactgacgacaacaatgaaaagaagaagataaggtcggtgattgtgaaagagacatagaggacacatgtaaggtggaaaatgtaagggcggaaagtaaccttatcacaaaggaatcttatcccccactacttatccttttatatttttccgtgtcatttttgcccttgagttttcctatataaggaaccaagttcggcatttgtgaaaacaagaaaaaatttggtgtaagctattttctttgaagtactgaggatacaacttcagagaaatttgtaagtttgtggatcctgcaggctagcgtgcactctagactcgacgaactgacgagctcgaatttccccgatcgttcaaacatttggcaataaagtttcttaagattgaatcctgttgccggtcttgcgatgattatcatataatttctgttgaattacgttaagcatgtaataattaacatgtaatgcatgacgttatttatgagatgggtttttatgattagagtcccgcaattatacatttaatacgcgatagaaaacaaaatatagcgcgcaaactatgataaattatcgcgcgcggtgtcatctatgttactagatcgggaattcctcgagcaactatttttatgtatgcaagagtcagcatatgtataattgattcagaatcgttttgacgagttcggatgtagtagtagccattatttaatgtacatactaatcgtgaatagtgaatatgatgaaacattgtatcttattgtataaatatccataaacacatcatgaaagacactttctttcacggtctgaattaattatgatacaattctaatagaaaacgaattaaattacgttgaattgtatgaaatctaattgaacaagccaaccacgacgacgactaacgttgcctggattgactcggtttaagttaaccactaaaaaaacggagctgtcatgtaacacgcggatcgagcaggtcacagtcatgaagccatcaaagcaaaagaactaatccaagggctgagatgattaattagtttaaaaattagttaacacgagggaaaaggctgtctgacagccaggtcacgttatctttacctgtggtcgaaatgattcgtgtctgtcgattttaattatttttttgaaaggccgaaaataaagttgtaagagataaacccgcctatataaattcatatattttcctctccgctttgaattgtctcgttgtcctcctcactttcatcagccgttttgaatctccggcgacttgacagagaagaacaaggaagaagactaagagagaaagtaagagataatccaggagattcattctccgttttgaatcttcctcaatctcatcttcttccgctctttctttccaaggtaataggaactttctggatctactttatttgctggatctcgatcttgttttctcaatttccttgagatctggaattcgtttaatttggatctgtgaacctccactaaatcttttggttttactagaatcgatctaagttgaccgatcagttagctcgattatagctaccagaatttggcttgaccttgatggagagatccatgttcatgttacctgggaaatgatttgtatatgtgaattgaaatctgaactgttgaagttagattgaatctgaacactgtcaatgttagattgaatctgaacactgtttaaggttagatgaagtttgtgtatagattcttcgaaactttaggatttgtagtgtcgtacgttgaacagaaagctatttctgattcaatcagggtttatttgactgtattgaactctttttgtgtgtttgcagctcataaaaggtaccaaacaatgattgaacaagatggattgcacgcaggttctccggccgcttgggtggagaggctattcggctatgactgggcacaacagacaatcggctgctctgatgccgccgtgttccggctgtcagcgcaggggcgcccggttctttttgtcaagaccgacctgtccggtgccctgaatgaactgcaggacgaggcagcgcggctatcgtggctggccacgacgggcgttccttgcgcagctgtgctcgacgttgtcactgaagcgggaagggactggctgctattgggcgaagtgccggggcaggatctcctgtcatctcaccttgctcctgccgagaaagtatccatcatggctgatgcaatgcggcggctgcatacgcttgatccggctacctgcccattcgaccaccaagcgaaacatcgcatcgagcgagcacgtactcggatggaagccggtcttgtcgatcaggatgatctggacgaagagcatcaggggctcgcgccagccgaactgttcgccaggctcaaggcgcgcatgcccgacggcgaggatctcgtcgtgacccatggcgatgcctgcttgccgaatatcatggtggaaaatggccgcttttctggattcatcgactgtggccggctgggtgtggcggaccgctatcaggacatagcgttggctacccgtgatattgctgaagagcttggcggcgaatgggctgaccgcttcctcgtgctttacggtatcgccgctcccgattcgcagcgcatcgccttctatcgccttcttgacgagttcttttgagcgggactctggcgatcgccccgatcgttcaaacatttggcaataaagtttcttaagattgaatcctgttgccggtcttgcgatgattatcatataatttctgttgaattacgttaagcatgtaataattaacatgtaatgcatgacgttatttatgagatgggtttttatgattagagtcccgcaattatacatttaatacgcgatagaaaacaaaatatagcgcgcaaactaggataaattatcgcgcgcggtgtcatctatgttactagatcgggactagt

SEQ ID NO: 32 - protein, 20 aa, Nicotiana tabacum
NGGGKTTSLGKLANRLKKEG

SEQ ID NO: 33 - protein, 23 aa, Nicotiana tabacum
RGGCVVSVVDELGIPVKFVGVGE

SEQ ID NO: 34 - protein, 20 aa, Nicotiana tabacum
KRGKGENVEYLVKWKDGEDN

SEQ ID NO: 35 - protein, 22 aa, Nicotiana tabacum
RTALLFVSGLGSEPCVKLLAEA

SEQ ID NO: 36 - protein, 20 aa, Nicotiana tabacum
RRSESRKQFADSGSTRPGPR

SEQ ID NO: 37 - protein, 18 aa, Nicotiana tabacum
LKEVKRVLNPTEVLLVVD

SEQ ID NO: 38 - DNA, 27 bp, Artificial Sequence
  source: /note="Description of Artificial Sequence: Synthetic primer"
atggcttctctattatcttctcgtctc

SEQ ID NO: 39 - DNA, 25 bp, Artificial Sequence
  source: /note="Description of Artificial Sequence: Synthetic primer"
gttcaaatgctcagctggtggaacg

SEQ ID NO: 40 - DNA, 25 bp, Artificial Sequence
  source: /note="Description of Artificial Sequence: Synthetic primer"
cgtcaattcctctctctcccgcctc

SEQ ID NO: 41 - DNA, 25 bp, Artificial Sequence
  source: /note="Description of Artificial Sequence: Synthetic primer"
cttcagaaccagcagcaacaagcag

SEQ ID NO: 42 - DNA, 26 bp, Artificial Sequence
  source: /note="Description of Artificial Sequence: Synthetic primer"
atggaagccactgcttctttctcctc

SEQ ID NO: 43 - DNA, 28 bp, Artificial Sequence
  source: /note="Description of Artificial Sequence: Synthetic primer"
ctcattcactagggatacatggagggtg

SEQ ID NO: 44 - protein, 6 aa, Artificial Sequence
  source: /note="Description of Artificial Sequence: Synthetic 6xHis tag"
HHHHHH

SEQ ID NO: 45 - DNA, 285 bp, Artificial Sequence
  source: /note="Description of Artificial Sequence: Synthetic polynucleotide"
ggatccatggcttctctattatcttctcgtctcccacgtcatctttcctctaataaaccggtactcccaccatcaagctccggttcaaatctccttcacaacttcacatataaaacccggttcgatcaatcccggttcaaatgctcagctggtggaacggggttcttcacgaagttgggtcgtttgctgaaagagaaagcaaagagcgacgtggagaaactgttctcaggattctcaaaaactcgagacaatttagcagttatagatgaactcctcctttactgg

SEQ ID NO: 46 - DNA, 153 bp, Artificial Sequence
  source: /note="Description of Artificial Sequence: Synthetic polynucleotide"
taataagatcttcaacacctacaccatttttttaatcactactacccattgcattgaacaaacttccaagttcttcttagcttcagattaagaaagtaccctttcttggctttgttgatgtggtaccattgtccattgtcttgtgtgtttcca

SEQ ID NO: 47 - DNA, 285 bp, Artificial Sequence
  source: /note="Description of Artificial Sequence: Synthetic polynucleotide"
ccagtaaaggaggagttcatctataactgctaaattgtctcgagtttttgagaatcctgagaacagtttctccacgtcgctctttgctttctctttcagcaaacgacccaacttcgtgaagaaccccgttccaccagctgagcatttgaaccgggattgatcgaaccgggttttatatgtgaagttgtgaaggagatttgaaccggagcttgatggtgggagtaccggtttattagaggaaagatgacgtgggagacgagaagataatagagaagccattctaga

SEQ ID NO: 48 - DNA, 306 bp, Artificial Sequence
  source: /note="Description of Artificial Sequence: Synthetic polynucleotide"
ggatccgggaaaggaatggagtacttgatagagtggaaagacgaacatgccccaacgtgggtcccctctgattacattgctaaagatgttgtggccgagtacgaaactccttggtggaatgcggctaaaaaggccgacgaatccgctcttagggaactcctagaaactgacgacgacagagatgtggacgcagtagatgaggatggacgtacggctttgctctttgtctcgggtctggggtccgagccgtgtgtcaagctgctagctgaagccggcgctgacgtggactatcgcgataggaatggc

SEQ ID NO: 49 - DNA, 153 bp, Artificial Sequence; identical to SEQ ID NO: 46
  source: /note="Description of Artificial Sequence: Synthetic polynucleotide"

SEQ ID NO: 50 - DNA, 306 bp, Artificial Sequence
  source: /note="Description of Artificial Sequence: Synthetic polynucleotide"
gccattcctatcgcgatagtccacgtcagcgccggcttcagctagcagcttgacacacggctcggaccccagacccgagacaaagagcaaagccgtacgtccatcctcatctactgcgtccacatctctgtcgtcgtcagtttctaggagttccctaagagcggattcgtcggcctttttagccgcattccaccaaggagtttcgtactcggccacaacatctttagcaatgtaatcagaggggacccacgttggggcatgttcgtctttccactctatcaagtactccattcctttccctctaga

SEQ ID NO: 51 - DNA, 297 bp, Artificial Sequence
  source: /note="Description of Artificial Sequence: Synthetic polynucleotide"
ggatccatggaagccactgcttctttctcctcaactatgtcttcccaccatttctttccactttccaaagccaccctctcaacttctaaacttccattttctgggactggttcaactcattctctttcattttcttcaagaaactcattcactagggatacatggagggtgatcaattcaaggaatgtggttatttcaagaagagaaatgcgtggagttattagagctgagatgtttggacagctcactagtggacttgaatcagcttggaataagctcaaaggagaagaggttttg

SEQ ID NO: 52 - DNA, 153 bp, Artificial Sequence; identical to SEQ ID NO: 46
  source: /note="Description of Artificial Sequence: Synthetic polynucleotide"

SEQ ID NO: 53 - DNA, 297 bp, Artificial Sequence
  source: /note="Description of Artificial Sequence: Synthetic polynucleotide"
caaaacctcttctcctttgagcttattccaagctgattcaagtccactagtgagctgtccaaacatctcagctctaataactccacgcatttctcttcttgaaataaccacattccttgaattgatcaccctccatgtatccctagtgaatgagtttcttgaagaaaatgaaagagaatgagttgaaccagtcccagaaaatggaagtttagaagttgagagggtggctttggaaagtggaaagaaatggtgggaagacatagttgaggagaaagaagcagtggcttccattctaga

SEQ ID NO: 54 - DNA, 417 bp, Artificial Sequence
  source: /note="Description of Artificial Sequence: Synthetic polynucleotide"
ggatccgaggcaggtgagttaacaaacaagaaaagctcctggttgacactctttgatgtggaagatccaaggtcaaaatttcctcagtctaaaggcaagttcctggatgcaaatcaagctttagaagttgctagatttgatatacaatattgtgattggcgagctcggcaagatgtattaaccataatgctcctgcacgaaaaggttgtggaagtattgaatcctctggcacgtgagtacaaatctattggaaccatgaaaaaggaacttgcagagttgcaaggagagctttctcaggcccacaaccaggtacatatatctgaggcccgggtttctgctgctttggataagctagcttacatggaagagttggttaatgataggcttctgcaagagagaagcacggcagaatcagat

SEQ ID NO: 55 - DNA, 153 bp, Artificial Sequence; identical to SEQ ID NO: 46
  source: /note="Description of Artificial Sequence: Synthetic polynucleotide"

SEQ ID NO: 56 - DNA, 417 bp, Artificial Sequence
  source: /note="Description of Artificial Sequence: Synthetic polynucleotide"
atctgattctgccgtgcttctctcttgcagaagcctatcattaaccaactcttccatgtaagctagcttatccaaagcagcagaaacccgggcctcagatatatgtacctggttgtgggcctgagaaagctctccttgcaactctgcaagttcctttttcatggttccaatagatttgtactcacgtgccagaggattcaatacttccacaaccttttcgtgcaggagcattatggttaatacatcttgccgagctcgccaatcacaatattgtatatcaaatctagcaacttctaaagcttgatttgcatccaggaacttgcctttagactgaggaaattttgaccttggatcttccacatcaaagagtgtcaaccaggagcttttcttgtttgttaactcacctgcctctctaga